European Patent Specification EP 3 811 777 B1, published July 31, 2024. Title: Genetically modified non-human animals. Applicant: Shanghai RAAS Blood Products Co., Ltd. The sequence listing filed with the application follows.

SEQUENCE LISTING (36 sequences)

SEQ ID NO: 1 - DNA, 17617 bp, Artificial Sequence
  Nucleotide sequence of targeting vector
cgcttacaatttccattcgccattcaggctgcgcaactgttgggaagggcgatcggtgcgggcctcttcgctattacgccagctggcgaaagggggatgtgctgcaaggcgattaagttgggtaacgccagggttttcccagtcacgacgttgtaaaacgacggccagtgaattgtaatacgactcactatagggcgaattggagctccaccgcccgggctggttctttccgcctcagaagccatagagcccaccgcatccccagcatgcctgctattgtcttcccaatcctcccccttgctgtcctgccccaccccaccccccagaatagaatgacacctactcagacaatgcgatgcaatttcctcattttattaggaaaggacagtgggagtggcaccttccagggtcaaggaaggcacgggggaggggcaaacaacagatggctggcaactagaaggcacagtcgaggctgatcagcgagctctaggatctgcattccaccactgctcccattcatcagttccataggttggaatctaaaatacacaaacaattagaatcagtagtttaacacattatacacttaaaaattttatatttaccttagagctttaaatctctgtaggtagtttgtccaattatgtcacaccacagaagtaaggttccttcacaaagagatcgcctgacacgatttcctgcacaggcttgagccatatactcatacatcgcatcttggccacgttttccacgggtttcaaaattaatctcaagttctacgcttaacgctttcgcctgttcccagttattaatatattcaacgctagaactcccctcagcgaagggaaggctgagcactacacgcgaagcaccatcaccgaaccttttgataaactcttccgttccgacttgctccatcaacggttcagtgagacttaaacctaactctttcttaatagtttcggcattatccacttttagtgcgagaaccttcgtcagtcctggatacgtcactttgaccacgcctccagcttttccagagagcgggttttcattatctacagagtatcccgcagcgtcgtatttattgtcggtactataaaaccctttccaatcatcgtcataatttccttgtgtaccagattttggcttttgtatacctttttgaatggaatctacataaccaggtttagtcccgtggtacgaagaaaagttttccatcacaaaagatttagaagaatcaacaacatcatcaggatccatggcacgcgcttctacaaggcgctggccgaagaggtgcgggagtttcacgccaccaagatctgcggcacgctgttgacgctgttaagcgggtcgctgcagggtcgctcggtgttcgaggccacacgcgtcaccttaatatgcgaagtggacctgggaccgcgccgccccgactgcatctgcgtgttcgaattcgccaatgacaagacgctgggcggggtttgctcgacattgggtggaaacattccaggcctgggtggagaggctttttgcttcctcttgcaaaaccacactgctcgacattgggtggaaacattccaggcctgggtggagaggctttttgcttcctcttgaaaaccacactgctcgatttgttagcagcctcgaatcaacccgggcgatcctaggcgatgagatctagctgtcgcgaagagtggcgcgcctccctgcacagctagtcacaacgaaggaaggcgcttagggaaccctggcagcttgcaaaacgcaaagggctacggctgcatcgctcttttccagacttctcagctgggagcttctggcagttttcccgagtcactcctttctctcactagctcacaaagtggccagctgagtcagaagcctccttctagtacaggcctgcctcccaccaacgccatcaatcaggacaagtaaggaagacttctgagtcgccccccccccccaccggtcaaatagaggggacatcttatcactgatggcatcctagattggtgatatatgtaattatttttgagtgtgctacccacgaacaagctatatctgtttatggttgctgttgttttggtttttgttttcttttaaggttctcatccctcagccactgcgggcaaaaatgagaccacatttgccaataagtttgaacacgctcaaccctctctttctccctccctttctgatagacaattccttcggtaggcagaggtgagcaatgggcacacggagccttccagagctgggatcagaaaacctcttgtttgtttgtctggggagagggaggttcggcaccaagggctaagcaaatatttgcggttatggattaacctgactcccagactgacatggcgctacctggacgaaattgcagtttctccttggcccacgcctgtaagtccccctcattgcaagactgtgaaggactgtggagggaggggaggggaggaaagtccagctgggaggaaggtgacgttcttgagctaaggctctccaggcagactgaaatgtggggccaaggaaaatgagcgcccaaactctatctggaccaaggcgtgggttccctacaatccaggtgaccatctcgacacatgagattttgtggatcaagtggacagcagtcaaagggttccctatgatcaggaaccatcctcagagcaatcttgaaacccagaaccccactactcccctctgccctgttctctaaggtggactctacaattccggaagccagcaaagccgaagagtgaggccaggaggggctgtgcagctgggataggcgggcctgcccacctggtctgggggacactagaggccttgtggtttgactactggttgggggcaggggttaaggttccagagttggggccacataggcttggccttgaagccaaactctgccctcctcttaggtgtaggcttgtgacaagccgcgtatctcctccaagcctttgggtcccttcccatgaaatggaggtgagaatattcatgccttcctcttttaacagtgatcagtgtgtgtgtgtgtgtgtgtgtgtgtgtgtgtgtgtgtgtgtgtgtgtgtgtgtgtggtgtagagtgtggtttctggtgttcagggttgaacccagaatcttaaacatgccaagtacgttctttcctactgaactgcaaccctccagtatcctgtacttgttgtttgtttgtttgtttgtttgtttgttcggaagcacctgtggtggcacacacttacaatcctagtgctagagagcagaaacaagtggatcccttgggcttgctggctggccagcctacgtgatgagtttcaggcagtgagagaccttgtcccaaacaataaggtggaagtaagccatgatggcatacccctttagagctagtactcgagaggcagaagcaggtggagtttaagaccagcctggtctacatagaagttccaggatagccaaaaagtacccaaggccatccaaaaaaacaaaaacaaaacaaaacctggagggaaaaaaaaaaccagacaatgcctggggaaggatgaaggacagtcagtcagattatccctggtcaacacgtgtgcacaaatctgtgcacacaagaaagagcttcacatgggttactatttgttttccaacaactcatttttaagcccccactctctttctctgtttttaaaaaaggtttatttattttatgtatatgagtacattattgctctcttcagacacaccagaaaaggacataagattccattacagatggttgtgagccaccatgtggttgctggaatttgaactcaggtcctctggaagagcagtcggtgctcttaaccactgaaccatctccccagcccttccaacaactctttatggaagaaacctattctatccattttataaatgacagaactgaggcacggagcacgtaaacatcttgttaaatacctctctctctctctctctctccccagtaggaaatggaatttgccccaggcaatgacttttttttttttttttttgctttcatgtacctagagtaagcccagctctaaaggccacgagattgtctgtctgtggaccgtggtgtaccccactcccagacccagcttccacacagacaatgagctcacaaacgtcctttactcccttccttccttgcttgctctgtgtgtgtgtgtgtgtgtgtgtgtgtgtgttaagagatcaacctcagacattttctttaggagctatttaccttgctttttgagacagggcctccggatggcctggagctagtcacctggagctggtcaagcaggctagggtggctggcctaagcaatccacaggatctgcttatctctgcctccccagtcctgggattacaagaaacgcctcagacacctagatttctgttttaattttctatgggttctggggatctttcttaagtcttcaagtatgcacggaaagggctttattgactaagatatctcccctgctcaggaatggccctttcattctactttggagggagctgggggtggggcggggagcagctcagctgtgtgtatccttggagcttagaagttctcctcagacaggtgtcagcagctccaggatgtggcagctcacaagcctcctgctgttcgtggccacctggggaatttccggcacaccagctcctcttgactcagtgttctccagcagcgagcgtgcccaccaggtgctgcggatccgcaaacgtgccaactccttcctggaggagctccgtcacagcagcctggagcgggagtgcatagaggagatctgtgacttcgaggaggccaaggaaattttccaaaatgtggatgacacactggccttctggtccaagcacgtcgacggtgaccagtgcttggtcttgcccttggagcacccgtgcgccagcctgtgctgcgggcacggcacgtgcatcgacggcatcggcagcttcagctgcgactgccgcagcggctgggagggccgcttctgccagcgcgaggtgagcttcctcaattgctcgctggacaacggcggctgcacgcattactgcctagaggaggtgggctggcggcgctgtagctgtgcgcctggctacaagctgggggacgacctcctgcagtgtcaccccgcagtgaagttcccttgtgggaggccctggaagcggatggagaagaagcgcagtcacctgaaacgagacacagaagaccaagaagaccaagtagatccgcggctcattgatgggaagatgaccaggcggggagacagcccctggcaggtggtcctgctggactcaaagaagaagctggcctgcggggcagtgctcatccacccctcctgggtgctgacagcggcccactgcatggatgagtccaagaagctccttgtcaggcttggagagtatgacctgcggcgctgggagaagtgggagctggacctggacatcaaggaggtcttcgtccaccccaactacagcaagagcaccaccgacaatgacatcgcactgctgcacctggcccagcccgccaccctctcgcagaccatagtgcccatctgcctcccggacagcggccttgcagagcgcgagctcaatcaggccggccaggagaccctcgtgacgggctggggctaccacagcagccgagagaaggaggccaagagaaaccgcaccttcgtcctcaacttcatcaagattcccgtggtcccgcacaatgagtgcagcgaggtcatgagcaacatggtgtctgagaacatgctgtgtgcgggcatcctcggggaccggcaggatgcctgcgagggcgacagtggggggcccatggtcgcctccttccacggcacctggttcctggtgggcctggtgagctggggtgagggctgtgggctccttcacaactacggcgtttacaccaaagtcagccgctacctcgactggatccatgggcacatcagagacaaggaagccccccagaagagctgggcaccttagcacccctccctgctcacctctggaccctagaagtcactcttggagtaaggctgggctagtgagtaccaagacagaggacattaaaggagcatgcaacaaacatacctccccgagtacctgtctgtcttttcatcctttttatgggctattctgggggaaagtaacattaattgagcatgcactacacaccaagtctatgaaaagaacctgcttaactcccaaagcagttgtgtagaagatctagtgggatctgagctgatatcacttctgggggtgagtggaggagattgatttagagaaaggaatttttttagaagttactgtaagagactaatagagcctttctcagggccttggaaagagcccgtgctagttacatcagaaaagcttgccagtgaccagtggccagtgagactcagaatggccatgtggtggagccaggattcaaaccaaggtcacactcccaaactcagctgcttctcttctttattatccctgggtgtgtgctggtgtgtgtgtgcgcgcgtgggtgtgtgggtggatacatgcatgtgtgtgtgtgtgtgtgtgtgtgtgtgtgtgtgtgtgtgtgttatatgtttggagaccagaggacaacttcgtttctcaacaccatccacttgttttgttttgtgttttgttttgtttgttgacacagggtctctcactgtcctgaaatctacccagtaggctaggctggctggctaccaaaccccaccccaccctggctttgacaagtggagacagaagaccagtagtccactggagatgtgaccagatgcccagaaggtgctcctcatggtgccctacagttttgttgaggagtctgtttaataatgcagctgggtgcagtggcagcacctgtagcccccaatactgaggcagcattgctgcagtctgagaggtggggctcgagggacctaataacttcgtatagcatacattatacgaagttatattaagggttccgcaagctctagtcgagccccagctggttctttccgcctcagaagccatagagcccaccgcatccccagcatgcctgctattgtcttcccaatcctcccccttgctgtcctgccccaccccaccccccagaatagaatgacacctactcagacaatgcgatgcaatttcctcattttattaggaaaggacagtgggagtggcaccttccagggtcaaggaaggcacgggggaggggcaaacaacagatggctggcaactagaaggcacagtcgaggctgatcagcgagctctagagaattgatcccctcagaagaactcgtcaagaaggcgatagaaggcgatgcgctgcgaatcgggagcggcgataccgtaaagcacgaggaagcggtcagcccattcgccgccaagctcttcagcaatatcacgggtagccaacgctatgtcctgatagcggtccgccacacccagccggccacagtcgatgaatccagaaaagcggccattttccaccatgatattcggcaagcaggcatcgccatgggtcacgacgagatcatcgccgtcgggcatgcgcgccttgagcctggcgaacagttcggctggcgcgagcccctgatgctcttcgtccagatcatcctgatcgacaagaccggcttccatccgagtacgtgctcgctcgatgcgatgtttcgcttggtggtcgaatgggcaggtagccggatcaagcgtatgcagccgccgcattgcatcagccatgatggatactttctcggcaggagcaaggtgagatgacaggagatcctgccccggcacttcgcccaatagcagccagtcccttcccgcttcagtgacaacgtcgagcacagctgcgcaaggaacgcccgtcgtggccagccacgatagccgcgctgcctcgtcctgcagttcattcagggcaccggacaggtcggtcttgacaaaaagaaccgggcgcccctgcgctgacagccggaacacggcggcatcagagcagccgattgtctgttgtgcccagtcatagccgaatagcctctccacccaagcggccggagaacctgcgtgcaatccatcttgttcaatggccgatcccatggtttagttcctcaccttgtcgtattatactatgccgatatactatgccgatgattaattgtcaacaggctgcaggtcgaaaggcccggagatgaggaagaggagaacagcgcggcagacgtgcgcttttgaagcgtgcagaatgccgggcctccggaggaccttcgggcgcccgccccgcccctgagcccgcccctgagcccgcccccggacccaccccttcccagcctctgagcccagaaagcgaaggagcaaagctgctattggccgctgccccaaaggcctacccgcttccattgctcagcggtgctgtccatctgcacgagactagtgagacgtgctacttccatttgtcacgtcctgcacgacgcgagctgcggggcgggggggaacttcctgactaggggaggagtagaaggtggcgcgaaggggccaccaaagaacggagccggttggcgcctaccggtggatgtggaatgtgtgcgaggccagaggccacttgtgtagcgccaagtgcccagcggggctgctaaagcgcatgctccagactgccttgggaaaagcgcctcccctacccggtagaatttcgacgacctgcagccaagctagcttcgcgagctcgaccgaacaaacgacccaacacccgtgcgttttattctgtctttttattgccgctcagctttacagtgacaatgacggctggcgactgaatattagtgcttacagacagcactacatattttccgtcgatgttgaaatcctttctcatatgtcaccataaatatcaaataattatagcaatcatttacgcgttaatggctaatcgccatcttccagcaggcgcaccattgcccctgtttcactatccaggttacggatatagttcatgacaatatttacattggtccagccaccagcttgcatgatctccggtattgaaactccagcgcgggccatatctcgcgcggctccgacacgggcactgtgtccagaccaggccaggtatctctgaccagagtcatccttagcgccgtaaatcaatcgatgagttgcttcaaaaatcccttccagggcgcgagttgatagctggctggtggcagatggcgcggcaacaccattttttctgacccggcaaaacaggtagttattcggatcatcagctacaccagagacggaaatccatcgctcgaccagtttagttacccccaggctaagtgccttctctacacctgcggtgctaaccagcgttttcgttctgccaatatggattaacattctcccaccgtcagtacgtgagatatctttaaccctgatcctggcaatttcggctatacgtaacagggtgttataagcaatccccagaaatgccagattacgtatatcctggcagcgatcgctattttccatgagtgaacgaacctggtcgaaatcagtgcgttcgaacgctagagcctgttttgcacgttcaccggcatcaacgttttcttttcggatccgccgcataaccagtgaaacagcattgctgtcacttggtcgtggcagcccggaccgacgatgaagcatgtttagctggcccaaatgttgctggatagtttttactgccagaccgcgcgcctgaagatatagaagataatcgcgaacatcttcaggttctgcgggaaaccatttccggttattcaacttgcaccatgccgcccacgaccggcaaacggacagaagcattttccaggtatgctcagaaaacgcctggcgatccctgaacatgtccatcaggttcttgcgaacctcatcactcgttgcatcgaccggtaatgcaggcaaattttggtgtacggtcagtaaattggacaccttcctcttcttcttgggcatggccgcaggaaagcagagccctgaagctcccatcaccggccaataagagccaagcctgcagtgtgacctcatagagcaatgtgccagccagcctgaccccaagggccctcaggcttgggcacactgtctctaggaccctgagagaaagacatacccatttctgcttagggccctgaggatgagcccaggggtggcttggcactgaagcaaaggacactggggctcagctggcagcaaagtgaccaggatgctgaggctttgacccagaagccagaggccagaggccaggacttctcttggtcccagtccaccctcactcagagctttaccaatgccctctggatagttgtcgggtaacggtggacgccactgattctctggccagcctaggacttcgccattccgctgattctgctcttccagccactggctgaccggttggaagtactccagcagtgccttggcatccagggcatctgagcctaccaggtccttcagtacctcctgccagggcctggagcagccagcctgcaacacctgcctgccaagcagagtgaccactgtgggcacaggggacacagggtggggcccacaacagcaccattgtccacttgtccctcactagtaaaagaactctagggttgcggggggtgggggaggtctctgtgaggctggtaagggatatttgcctggcccatggagctagcttggctggacgtaaactcctcttcagacctaataacttcgtatagcatacattatacgaagttatattaagggttattgaatatgatcggaattgggctgcaggaattcgatagcttggctgcaggtcgacgtacgtagcaagcttgatgggccctggtaccacagcctgggcaacacagcaaaaatcccttcccttaaaaaaaacaaaagagaaggaagaaggacgaagtagaatgtggaggacaaacaggggagagagggggaaagaaagggagggaattgtcttagagttttacggctgtgcacagacaccatgatcaaggtaactcttgtaaggataacatttagttggggctggcttacaggttcagaagttcagtccattatcatcaaggcaggaacatggcagcattcaaggcagacatggtgcaggaggagctgagagttctacatcttcatctgaagatttctagtagaatactggcttccaggcagctaggatgagggtcttaaagcccacacccagtgacacacctactccaacagggccacacctcctaatcatgccactccctgggctgagcatatagaaaccatcacagagtctaactagtgtggcccatcctgcacccatggaagaccatcactggggcatagacaacctccagagcccaccctgacagttcctgtctctgccttctccagcagtcaccagtttcaaatagctcctcaaggacagatggggccttgtgagcttcaccccgctgcaggctggaatgcgccacctttaatcccagcacttggaaggcagaggcaggcagatttctgagttcgaggccagcctagtctacagagtgagttccaggacagccagggcgatacagagaaaccctgtctcaaaaaacaaaacaaaacaaaacgatagaaaagagcaaagtgaccttgggctatggatgggatggaccatcgggcactgggttgggaagctgaactggtccagatgcccagagcccagagctctctcctcagcagttcataacctggggtgttgccacagcacacacagcaaggttagttctgctggttgtcgggacttagggtaggaggagtagaagcctgctactgattctgtctctctctgtttctctctcctccctccctccctccttccctccctccctccctcttcttcttcttctcatcctcctccctcttcctcttcttcctccacctccccaccccttattttgatacagggtttctctgtgtatccctggctgtcctggaactcactctgtagcccaggtgggcctcgaactctcagcctcagtccccagaatgctgagaacacaggtctgagtgatcactgatggctaaaagttgggattacattgttgttgcttgtttgtttattcttttgtacatgggacccaaatacaaatagtagcctcaacaataaacacgggataagttgctgctctgctttagggtctccctgacctctgtttttttgttttttgtttttggtatgttttgttttctgttgttgttgttatcatgtctataaatctatcttccttcctccctccttccttcccttcctacttccctctctttcttcatccctcccttccccctactctctttcacccccagataggaagcaagcatgataaaaacgtgtggtgttttcctttttatgtagagagtactgtgtagtgagtgttatcctatgggtgctgccattctgctgtatgttacctgctgtatgttataccaacctagatggtggtgaactcacatggttgcttccatcttggtgaggttaccagccaagatgtctgccctccacatgattgcctccatcttggtgaggtaaatgtttaataaagtaacaaaacaagacattaaaaacaaacattccagcacaaaatcttcttgagattagagacataataggaagtcaggtgaggtcatacaggccattaatcccatcacttggggaacagaggcaggtagaactttgaattgaaggcaggtatatttagtgatttccagggctatgtagagaggcccctgacccaactaataagtaaacaggaagataaataaatataatgaacttagaataaaacaaagaaaggaagaaacaagggaaggcagtgctgggggcctggcttatggtggatgggggaattctgtgctagggtgcctgaaactctgggctccatcctctgtagtgcataaactctttggtacgttagcccctgtctgtaacaaggagctgtccacggttgcagtactgcctttcccatctcagctgcccctcaggagctgtccacagtggcgacactttttcatcctcagcctacagctttagggaaacaccactgcaggggctgtcccaaaggtgctgtccacagaggcagcaccttctctgtggtctcacccctccagacaccccccagcagccccacagggatggcacctcagtaaaagccaactgtggccagagaagtcttcctaccctaactcatagactcgatgcagggaaaacagggtgaaaaaaagccaccaagccctgagctccccccagctcaggacttaaaatctcatcaatcctcactatggaaatctctgccttgagaagctctgccccctcataaatcctatataagaactgtccctttgtccagttccctgccatccgctcccaggagcagagggcagttatccctggattcatccctccacaccctggacctgccaataaacctttcttgagatttcatgcttcctgtgattctcagtggaagaagccaagaagaaaagaaccaaagagagggagccaggctgaggctcctgagttcttcagctcagctgtggatacctgtgatggtttgtatatgctctgtccagggaatggcatgattagaaggtgtggccctgttgaagtaggtgtgtcactgtgggtgtgggctataagaccctcatcttaactgcatggaagtcattcttccactggcagccttcagatgaaaatgtagaactctcagctcctcctgcaccatgcctgcctagatgctgccctgctcccaccttgatgataatggactgaacctctgaacctgtaagccagccccaattaaatgttgttctttataagtcttgccttggttgtggtgtctgttcacagcagtaaaaccatgactaagacaatatcttctacttggagctgcaacaactctgctgaggaggcttcctctcagagctatatggttcctggtatctgtaaaattcccttctattgggacactttccaacctcagatctgtgtggttcctggcccctgtgtctcgggatgcccttccattagaacagcttctcccctcagagctgcatggttcctggacttctgagtcccaggagacccttccatctgagcagaaacacttacaggagcagagtcctccaacaccacggttttgttttgaaagaccaagaccaaccctcaggaggtttctggcaaaggcagattctaggtgcacctggaggagacctatagtgcaggaccatccgtcgtaggttgctaggcaccaatgggcaaaggtagggaagaaatcttaccagaagattctattccattccattctcctcacaatgtaagagccaaagttaacctctaaggcccaagaacaaggtaactctccagaatgctgggagatgtagttcttgggtaacaacaagccatgttctcgccctaaacaagtttgtttgaatcaactacactgaatgtacttgatcatatgtaggagagagaagattgattctagttcagggtttcaggctatttcagtccaccatgatgggaaaggcatgacattgtttatgacagtaagagcatgtagcagaggatcctcacatcacaacaggccgaaatgcagaggacagtgcaaccagaggacagtctgtaactttccaagtccctcttctagtgggttgcttccaccacctctcaggtggtgctacagctcaggaacaattgagatgtgtgatgaagggcaggtactcaactgtggctgtattgtatccttttatagttgtcctctgtgtgttgagctatgtgcgagattctcaggtcatcggagtacctgttttactttggcaggcataggagactcctgagaactctgcctgacatccttgccagcccaagctttggtttagtgtgtgcagtatcactcttgggtcttatctgcatatccctgatggcccatcaagatgtgtgcggccgcgtaccagcttttgttccctttagtgagggttaatttcgagcttggcgtaatcatggtcatagctgtttcctgtgtgaaattgttatccgctcacaattccacacaacatacgagccggaagcataaagtgtaaagcctggggtgcctaatgagtgagctaactcacattaattgcgttgcgctcactgcccgctttccagtcgggaaacctgtcgtgccagctgcattaatgaatcggccaacgcgcggggagaggcggtttgcgtattgggcgctcttccgcttcctcgctcactgactcgctgcgctcggtcgttcggctgcggcgagcggtatcagctcactcaaaggcggtaatacggttatccacagaatcaggggataacgcaggaaagaacatgtgagcaaaaggccagcaaaaggccaggaaccgtaaaaaggccgcgttgctggcgtttttccataggctccgcccccctgacgagcatcacaaaaatcgacgctcaagtcagaggtggcgaaacccgacaggactataaagataccaggcgtttccccctggaagctccctcgtgcgctctcctgttccgaccctgccgcttaccggatacctgtccgcctttctcccttcgggaagcgtggcgctttctcatagctcacgctgtaggtatctcagttcggtgtaggtcgttcgctccaagctgggctgtgtgcacgaaccccccgttcagcccgaccgctgcgccttatccggtaactatcgtcttgagtccaacccggtaagacacgacttatcgccactggcagcagccactggtaacaggattagcagagcgaggtatgtaggcggtgctacagagttcttgaagtggtggcctaactacggctacactagaagaacagtatttggtatctgcgctctgctgaagccagttaccttcggaaaaagagttggtagctcttgatccggcaaacaaaccaccgctggtagcggtggtttttttgtttgcaagcagcagattacgcgcagaaaaaaaggatctcaagaagatcctttgatcttttctacggggtctgacgctcagtggaacgaaaactcacgttaagggattttggtcatgagattatcaaaaaggatcttcacctagatccttttaaattaaaaatgaagttttaaatcaatctaaagtatatatgagtaaacttggtctgacagttaccaatgcttaatcagtgaggcacctatctcagcgatctgtctatttcgttcatccatagttgcctgactccccgtcgtgtagataactacgatacgggagggcttaccatctggccccagtgctgcaatgataccgcgagacccacgctcaccggctccagatttatcagcaataaaccagccagccggaagggccgagcgcagaagtggtcctgcaactttatccgcctccatccagtctattaattgttgccgggaagctagagtaagtagttcgccagttaatagtttgcgcaacgttgttgccattgctacaggcatcgtggtgtcacgctcgtcgtttggtatggcttcattcagctccggttcccaacgatcaaggcgagttacatgatcccccatgttgtgcaaaaaagcggttagctccttcggtcctccgatcgttgtcagaagtaagttggccgcagtgttatcactcatggttatggcagcactgcataattctcttactgtcatgccatccgtaagatgcttttctgtgactggtgagtactcaaccaagtcattctgagaatagtgtatgcggcgaccgagttgctcttgcccggcgtcaatacgggataataccgcgccacatagcagaactttaaaagtgctcatcattggaaaacgttcttcggggcgaaaactctcaaggatcttaccgctgttgagatccagttcgatgtaacccactcgtgcacccaactgatcttcagcatcttttactttcaccagcgtttctgggtgagcaaaaacaggaaggcaaaatgccgcaaaaaagggaataagggcgacacggaaatgttgaatactcatactcttcctttttcaatattattgaagcatttatcagggttattgtctcatgagcggatacatatttgaatgtatttagaaaaataaacaaataggggttccgcgcacatttccccgaaaagtgccacctgacgcgccctgtagcggcgcattaagcgcggcgggtgtggtggttacgcgcagcgtgaccgctacacttgccagcgccctagcgcccgctcctttcgctttcttcccttcctttctcgccacgttcgccggctttccccgtcaagctctaaatcgggggctccctttagggttccgatttagtgctttacggcacctcgaccccaaaaaacttgattagggtgatggttcacgtagtgggccatcgccctgatagacggtttttcgccctttgacgttggagtccacgttctttaatagtggactcttgttccaaactggaacaacactcaaccctatctcggtctattcttttgatttataagggattttgccgatttcggcctattggttaaaaaatgagctgatttaacaaaaatttaacgcgaattttaacaaaatattaa

SEQ ID NO: 2 - DNA, 2901 bp, Artificial Sequence
  5' homology arm of targeting vector
tccctgcacagctagtcacaacgaaggaaggcgcttagggaaccctggcagcttgcaaaacgcaaagggctacggctgcatcgctcttttccagacttctcagctgggagcttctggcagttttcccgagtcactcctttctctcactagctcacaaagtggccagctgagtcagaagcctccttctagtacaggcctgcctcccaccaacgccatcaatcaggacaagtaaggaagacttctgagtcgccccccccccccaccggtcaaatagaggggacatcttatcactgatggcatcctagattggtgatatatgtaattatttttgagtgtgctacccacgaacaagctatatctgtttatggttgctgttgttttggtttttgttttcttttaaggttctcatccctcagccactgcgggcaaaaatgagaccacatttgccaataagtttgaacacgctcaaccctctctttctccctccctttctgatagacaattccttcggtaggcagaggtgagcaatgggcacacggagccttccagagctgggatcagaaaacctcttgtttgtttgtctggggagagggaggttcggcaccaagggctaagcaaatatttgcggttatggattaacctgactcccagactgacatggcgctacctggacgaaattgcagtttctccttggcccacgcctgtaagtccccctcattgcaagactgtgaaggactgtggagggaggggaggggaggaaagtccagctgggaggaaggtgacgttcttgagctaaggctctccaggcagactgaaatgtggggccaaggaaaatgagcgcccaaactctatctggaccaaggcgtgggttccctacaatccaggtgaccatctcgacacatgagattttgtggatcaagtggacagcagtcaaagggttccctatgatcaggaaccatcctcagagcaatcttgaaacccagaaccccactactcccctctgccctgttctctaaggtggactctacaattccggaagccagcaaagccgaagagtgaggccaggaggggctgtgcagctgggataggcgggcctgcccacctggtctgggggacactagaggccttgtggtttgactactggttgggggcaggggttaaggttccagagttggggccacataggcttggccttgaagccaaactctgccctcctcttaggtgtaggcttgtgacaagccgcgtatctcctccaagcctttgggtcccttcccatgaaatggaggtgagaatattcatgccttcctcttttaacagtgatcagtgtgtgtgtgtgtgtgtgtgtgtgtgtgtgtgtgtgtgtgtgtgtgtgtgtgtgtggtgtagagtgtggtttctggtgttcagggttgaacccagaatcttaaacatgccaagtacgttctttcctactgaactgcaaccctccagtatcctgtacttgttgtttgtttgtttgtttgtttgtttgttcggaagcacctgtggtggcacacacttacaatcctagtgctagagagcagaaacaagtggatcccttgggcttgctggctggccagcctacgtgatgagtttcaggcagtgagagaccttgtcccaaacaataaggtggaagtaagccatgatggcatacccctttagagctagtactcgagaggcagaagcaggtggagtttaagaccagcctggtctacatagaagttccaggatagccaaaaagtacccaaggccatccaaaaaaacaaaaacaaaacaaaacctggagggaaaaaaaaaaccagacaatgcctggggaaggatgaaggacagtcagtcagattatccctggtcaacacgtgtgcacaaatctgtgcacacaagaaagagcttcacatgggttactatttgttttccaacaactcatttttaagcccccactctctttctctgtttttaaaaaaggtttatttattttatgtatatgagtacattattgctctcttcagacacaccagaaaaggacataagattccattacagatggttgtgagccaccatgtggttgctggaatttgaactcaggtcctctggaagagcagtcggtgctcttaaccactgaaccatctccccagcccttccaacaactctttatggaagaaacctattctatccattttataaatgacagaactgaggcacggagcacgtaaacatcttgttaaatacctctctctctctctctctctccccagtaggaaatggaatttgccccaggcaatgacttttttttttttttttttgctttcatgtacctagagtaagcccagctctaaaggccacgagattgtctgtctgtggaccgtggtgtaccccactcccagacccagcttccacacagacaatgagctcacaaacgtcctttactcccttccttccttgcttgctctgtgtgtgtgtgtgtgtgtgtgtgtgtgtgttaagagatcaacctcagacattttctttaggagctatttaccttgctttttgagacagggcctccggatggcctggagctagtcacctggagctggtcaagcaggctagggtggctggcctaagcaatccacaggatctgcttatctctgcctccccagtcctgggattacaagaaacgcctcagacacctagatttctgttttaattttctatgggttctggggatctttcttaagtcttcaagtatgcacggaaagggctttattgactaagatatctcccctgctcaggaatggccctttcattctactttggagggagctgggggtggggcggggagcagctcagctgtgtgtatccttggagcttagaagttctcctcagacaggtgtcagcagctccagg

SEQ ID NO: 3 - DNA, 931 bp, Artificial Sequence
  First part of (i.e. 5' portion of) 3' homology arm of targeting vector
cacccctccctgctcacctctggaccctagaagtcactcttggagtaaggctgggctagtgagtaccaagacagaggacattaaaggagcatgcaacaaacatacctccccgagtacctgtctgtcttttcatcctttttatgggctattctgggggaaagtaacattaattgagcatgcactacacaccaagtctatgaaaagaacctgcttaactcccaaagcagttgtgtagaagatctagtgggatctgagctgatatcacttctgggggtgagtggaggagattgatttagagaaaggaatttttttagaagttactgtaagagactaatagagcctttctcagggccttggaaagagcccgtgctagttacatcagaaaagcttgccagtgaccagtggccagtgagactcagaatggccatgtggtggagccaggattcaaaccaaggtcacactcccaaactcagctgcttctcttctttattatccctgggtgtgtgctggtgtgtgtgtgcgcgcgtgggtgtgtgggtggatacatgcatgtgtgtgtgtgtgtgtgtgtgtgtgtgtgtgtgtgtgtgtgttatatgtttggagaccagaggacaacttcgtttctcaacaccatccacttgttttgttttgtgttttgttttgtttgttgacacagggtctctcactgtcctgaaatctacccagtaggctaggctggctggctaccaaaccccaccccaccctggctttgacaagtggagacagaagaccagtagtccactggagatgtgaccagatgcccagaaggtgctcctcatggtgccctacagttttgttgaggagtctgtttaataatgcagctgggtgcagtggcagcacctgtagcccccaatactgaggcagcattgctgcagtctgagaggtgggg

SEQ ID NO: 4 - DNA, 4126 bp, Artificial Sequence
  Second part of (i.e. 3' portion of) 3' homology arm of targeting vector
acagcctgggcaacacagcaaaaatcccttcccttaaaaaaaacaaaagagaaggaagaaggacgaagtagaatgtggaggacaaacaggggagagagggggaaagaaagggagggaattgtcttagagttttacggctgtgcacagacaccatgatcaaggtaactcttgtaaggataacatttagttggggctggcttacaggttcagaagttcagtccattatcatcaaggcaggaacatggcagcattcaaggcagacatggtgcaggaggagctgagagttctacatcttcatctgaagatttctagtagaatactggcttccaggcagctaggatgagggtcttaaagcccacacccagtgacacacctactccaacagggccacacctcctaatcatgccactccctgggctgagcatatagaaaccatcacagagtctaactagtgtggcccatcctgcacccatggaagaccatcactggggcatagacaacctccagagcccaccctgacagttcctgtctctgccttctccagcagtcaccagtttcaaatagctcctcaaggacagatggggccttgtgagcttcaccccgctgcaggctggaatgcgccacctttaatcccagcacttggaaggcagaggcaggcagatttctgagttcgaggccagcctagtctacagagtgagttccaggacagccagggcgatacagagaaaccctgtctcaaaaaacaaaacaaaacaaaacgatagaaaagagcaaagtgaccttgggctatggatgggatggaccatcgggcactgggttgggaagctgaactggtccagatgcccagagcccagagctctctcctcagcagttcataacctggggtgttgccacagcacacacagcaaggttagttctgctggttgtcgggacttagggtaggaggagtagaagcctgctactgattctgtctctctctgtttctctctcctccctccctccctccttccctccctccctccctcttcttcttcttctcatcctcctccctcttcctcttcttcctccacctccccaccccttattttgatacagggtttctctgtgtatccctggctgtcctggaactcactctgtagcccaggtgggcctcgaactctcagcctcagtccccagaatgctgagaacacaggtctgagtgatcactgatggctaaaagttgggattacattgttgttgcttgtttgtttattcttttgtacatgggacccaaatacaaatagtagcctcaacaataaacacgggataagttgctgctctgctttagggtctccctgacctctgtttttttgttttttgtttttggtatgttttgttttctgttgttgttgttatcatgtctataaatctatcttccttcctccctccttccttcccttcctacttccctctctttcttcatccctcccttccccctactctctttcacccccagataggaagcaagcatgataaaaacgtgtggtgttttcctttttatgtagagagtactgtgtagtgagtgttatcctatgggtgctgccattctgctgtatgttacctgctgtatgttataccaacctagatggtggtgaactcacatggttgcttccatcttggtgaggttaccagccaagatgtctgccctccacatgattgcctccatcttggtgaggtaaatgtttaataaagtaacaaaacaagacattaaaaacaaacattccagcacaaaatcttcttgagattagagacataataggaagtcaggtgaggtcatacaggccattaatcccatcacttggggaacagaggcaggtagaactttgaattgaaggcaggtatatttagtgatttccagggctatgtagagaggcccctgacccaactaataagtaaacaggaagataaataaatataatgaacttagaataaaacaaagaaaggaagaaacaagggaaggcagtgctgggggcctggcttatggtggatgggggaattctgtgctagggtgcctgaaactctgggctccatcctctgtagtgcataaactctttggtacgttagcccctgtctgtaacaaggagctgtccacggttgcagtactgcctttcccatctcagctgcccctcaggagctgtccacagtggcgacactttttcatcctcagcctacagctttagggaaacaccactgcaggggctgtcccaaaggtgctgtccacagaggcagcaccttctctgtggtctcacccctccagacaccccccagcagccccacagggatggcacctcagtaaaagccaactgtggccagagaagtcttcctaccctaactcatagactcgatgcagggaaaacagggtgaaaaaaagccaccaagccctgagctccccccagctcaggacttaaaatctcatcaatcctcactatggaaatctctgccttgagaagctctgccccctcataaatcctatataagaactgtccctttgtccagttccctgccatccgctcccaggagcagagggcagttatccctggattcatccctccacaccctggacctgccaataaacctttcttgagatttcatgcttcctgtgattctcagtggaagaagccaagaagaaaagaaccaaagagagggagccaggctgaggctcctgagttcttcagctcagctgtggatacctgtgatggtttgtatatgctctgtccagggaatggcatgattagaaggtgtggccctgttgaagtaggtgtgtcactgtgggtgtgggctataagaccctcatcttaactgcatggaagtcattcttccactggcagccttcagatgaaaatgtagaactctcagctcctcctgcaccatgcctgcctagatgctgccctgctcccaccttgatgataatggactgaacctctgaacctgtaagccagccccaattaaatgttgttctttataagtcttgccttggttgtggtgtctgttcacagcagtaaaaccatgactaagacaatatcttctacttggagctgcaacaactctgctgaggaggcttcctctcagagctatatggttcctggtatctgtaaaattcccttctattgggacactttccaacctcagatctgtgtggttcctggcccctgtgtctcgggatgcccttccattagaacagcttctcccctcagagctgcatggttcctggacttctgagtcccaggagacccttccatctgagcagaaacacttacaggagcagagtcctccaacaccacggttttgttttgaaagaccaagaccaaccctcaggaggtttctggcaaaggcagattctaggtgcacctggaggagacctatagtgcaggaccatccgtcgtaggttgctaggcaccaatgggcaaaggtagggaagaaatcttaccagaagattctattccattccattctcctcacaatgtaagagccaaagttaacctctaaggcccaagaacaaggtaactctccagaatgctgggagatgtagttcttgggtaacaacaagccatgttctcgccctaaacaagtttgtttgaatcaactacactgaatgtacttgatcatatgtaggagagagaagattgattctagttcagggtttcaggctatttcagtccaccatgatgggaaaggcatgacattgtttatgacagtaagagcatgtagcagaggatcctcacatcacaacaggccgaaatgcagaggacagtgcaaccagaggacagtctgtaactttccaagtccctcttctagtgggttgcttccaccacctctcaggtggtgctacagctcaggaacaattgagatgtgtgatgaagggcaggtactcaactgtggctgtattgtatccttttatagttgtcctctgtgtgttgagctatgtgcgagattctcaggtcatcggagtacctgttttactttggcaggcataggagactcctgagaactctgcctgacatccttgccagcccaagctttggtttagtgtgtgcagtatcactcttgggtcttatctgcatatccctgatggcccatcaagatgtgt

SEQ ID NO: 5 - DNA, 21 bp, Mouse
acaggtgtcagcagctccagg

SEQ ID NO: 6 - DNA, 104 bp, Mouse
cacccctccctgctcacctctggaccctagaagtcactcttggagtaaggctgggctagtgagtaccaagacagaggacattaaaggagcatgcaacaaacata

SEQ ID NO: 7 - DNA, 34 bp, Artificial Sequence
  LoxP site
ataacttcgtatagcatacattatacgaagttat

SEQ ID NO: 8 - DNA, 1386 bp, Human
atgtggcagctcacaagcctcctgctgttcgtggccacctggggaatttccggcacaccagctcctcttgactcagtgttctccagcagcgagcgtgcccaccaggtgctgcggatccgcaaacgtgccaactccttcctggaggagctccgtcacagcagcctggagcgggagtgcatagaggagatctgtgacttcgaggaggccaaggaaattttccaaaatgtggatgacacactggccttctggtccaagcacgtcgacggtgaccagtgcttggtcttgcccttggagcacccgtgcgccagcctgtgctgcgggcacggcacgtgcatcgacggcatcggcagcttcagctgcgactgccgcagcggctgggagggccgcttctgccagcgcgaggtgagcttcctcaattgctcgctggacaacggcggctgcacgcattactgcctagaggaggtgggctggcggcgctgtagctgtgcgcctggctacaagctgggggacgacctcctgcagtgtcaccccgcagtgaagttcccttgtgggaggccctggaagcggatggagaagaagcgcagtcacctgaaacgagacacagaagaccaagaagaccaagtagatccgcggctcattgatgggaagatgaccaggcggggagacagcccctggcaggtggtcctgctggactcaaagaagaagctggcctgcggggcagtgctcatccacccctcctgggtgctgacagcggcccactgcatggatgagtccaagaagctccttgtcaggcttggagagtatgacctgcggcgctgggagaagtgggagctggacctggacatcaaggaggtcttcgtccaccccaactacagcaagagcaccaccgacaatgacatcgcactgctgcacctggcccagcccgccaccctctcgcagaccatagtgcccatctgcctcccggacagcggccttgcagagcgcgagctcaatcaggccggccaggagaccctcgtgacgggctggggctaccacagcagccgagagaaggaggccaagagaaaccgcaccttcgtcctcaacttcatcaagattcccgtggtcccgcacaatgagtgcagcgaggtcatgagcaacatggtgtctgagaacatgctgtgtgcgggcatcctcggggaccggcaggatgcctgcgagggcgacagtggggggcccatggtcgcctccttccacggcacctggttcctggtgggcctggtgagctggggtgagggctgtgggctccttcacaactacggcgtttacaccaaagtcagccgctacctcgactggatccatgggcacatcagagacaaggaagccccccagaagagctgggcaccttag

SEQ ID NO: 9 - DNA, 13254 bp, Artificial Sequence
  Section of targeting vector from the 5' end of the 5' homology arm to the 3' end of the 3' homology arm
tccctgcacagctagtcacaacgaaggaaggcgcttagggaaccctggcagcttgcaaaacgcaaagggctacggctgcatcgctcttttccagacttctcagctgggagcttctggcagttttcccgagtcactcctttctctcactagctcacaaagtggccagctgagtcagaagcctccttctagtacaggcctgcctcccaccaacgccatcaatcaggacaagtaaggaagacttctgagtcgccccccccccccaccggtcaaatagaggggacatcttatcactgatggcatcctagattggtgatatatgtaattatttttgagtgtgctacccacgaacaagctatatctgtttatggttgctgttgttttggtttttgttttcttttaaggttctcatccctcagccactgcgggcaaaaatgagaccacatttgccaataagtttgaacacgctcaaccctctctttctccctccctttctgatagacaattccttcggtaggcagaggtgagcaatgggcacacggagccttccagagctgggatcagaaaacctcttgtttgtttgtctggggagagggaggttcggcaccaagggctaagcaaatatttgcggttatggattaacctgactcccagactgacatggcgctacctggacgaaattgcagtttctccttggcccacgcctgtaagtccccctcattgcaagactgtgaaggactgtggagggaggggaggggaggaaagtccagctgggaggaaggtgacgttcttgagctaaggctctccaggcagactgaaatgtggggccaaggaaaatgagcgcccaaactctatctggaccaaggcgtgggttccctacaatccaggtgaccatctcgacacatgagattttgtggatcaagtggacagcagtcaaagggttccctatgatcaggaaccatcctcagagcaatcttgaaacccagaaccccactactcccctctgccctgttctctaaggtggactctacaattccggaagccagcaaagccgaagagtgaggccaggaggggctgtgcagctgggataggcgggcctgcccacctggtctgggggacactagaggccttgtggtttgactactggttgggggcaggggttaaggttccagagttggggccacataggcttggccttgaagccaaactctgccctcctcttaggtgtaggcttgtgacaagccgcgtatctcctccaagcctttgggtcccttcccatgaaatggaggtgagaatattcatgccttcctcttttaacagtgatcagtgtgtgtgtgtgtgtgtgtgtgtgtgtgtgtgtgtgtgtgtgtgtgtgtgtgtgtggtgtagagtgtggtttctggtgttcagggttgaacccagaatcttaaacatgccaagtacgttctttcctactgaactgcaaccctccagtatcctgtacttgttgtttgtttgtttgtttgtttgtttgttcggaagcacctgtggtggcacacacttacaatcctagtgctagagagcagaaacaagtggatcccttgggcttgctggctggccagcctacgtgatgagtttcaggcagtgagagaccttgtcccaaacaataaggtggaagtaagccatgatggcatacccctttagagctagtactcgagaggcagaagcaggtggagtttaagaccagcctggtctacatagaagttccaggatagccaaaaagtacccaaggccatccaaaaaaacaaaaacaaaacaaaacctggagggaaaaaaaaaaccagacaatgcctggggaaggatgaaggacagtcagtcagattatccctggtcaacacgtgtgcacaaatctgtgcacacaagaaagagcttcacatgggttactatttgttttccaacaactcatttttaagcccccactctctttctctgtttttaaaaaaggtttatttattttatgtatatgagtacattattgctctcttcagacacaccagaaaaggacataagattccattacagatggttgtgagccaccatgtggttgctggaatttgaactcaggtcctctggaagagcagtcggtgctcttaaccactgaaccatctccccagcccttccaacaactctttatggaagaaacctattctatccattttataaatgacagaactgaggcacggagcacgtaaacatcttgttaaatacctctctctctctctctctctccccagtaggaaatggaatttgccccaggcaatgacttttttttttttttttttgctttcatgtacctagagtaagcccagctctaaaggccacgagattgtctgtctgtggaccgtggtgtaccccactcccagacccagcttccacacagacaatgagctcacaaacgtcctttactcccttccttccttgcttgctctgtgtgtgtgtgtgtgtgtgtgtgtgtgtgttaagagatcaacctcagacattttctttaggagctatttaccttgctttttgagacagggcctccggatggcctggagctagtcacctggagctggtcaagcaggctagggtggctggcctaagcaatccacaggatctgcttatctctgcctccccagtcctgggattacaagaaacgcctcagacacctagatttctgttttaattttctatgggttctggggatctttcttaagtcttcaagtatgcacggaaagggctttattgactaagatatctcccctgctcaggaatggccctttcattctactttggagggagctgggggtggggcggggagcagctcagctgtgtgtatccttggagcttagaagttctcctcagacaggtgtcagcagctccaggatgtggcagctcacaagcctcctgctgttcgtggccacctggggaatttccggcacaccagctcctcttgactcagtgttctccagcagcgagcgtgcccaccaggtgctgcggatccgcaaacgtgccaactccttcctggaggagctccgtcacagcagcctggagcgggagtgcatagaggagatctgtgacttcgaggaggccaaggaaattttccaaaatgtggatgacacactggccttctggtccaagcacgtcgacggtgaccagtgcttggtcttgcccttggagcacccgtgcgccagcctgtgctgcgggcacggcacgtgcatcgacggcatcggcagcttcagctgcgactgccgcagcggctgggagggccgcttctgccagcgcgaggtgagcttcctcaattgctcgctggacaacggcggctgcacgcattactgcctagaggaggtgggctggcggcgctgtagctgtgcgcctggctacaagctgggggacgacctcctgcagtgtcaccccgcagtgaagttcccttgtgggaggccctggaagcggatggagaagaagcgcagtcacctgaaacgagacacagaagaccaagaagaccaagtagatccgcggctcattgatgggaagatgaccaggcggggagacagcccctggcaggtggtcctgctggactcaaagaagaagctggcctgcggggcagtgctcatccacccctcctgggtgctgacagcggcccactgcatggatgagtccaagaagctccttgtcaggcttggagagtatgacctgcggcgctgggagaagtgggagctggacctggacatcaaggaggtcttcgtccaccccaactacagcaagagcaccaccgacaatgacatcgcactgctgcacctggcccagcccgccaccctctcgcagaccatagtgcccatctgcctcccggacagcggccttgcagagcgcgagctcaatcaggccggccaggagaccctcgtgacgggctggggctaccacagcagccgagagaaggaggccaagagaaaccgcaccttcgtcctcaacttcatcaagattcccgtggtcccgcacaatgagtgcagcgaggtcatgagcaacatggtgtctgagaacatgctgtgtgcgggcatcctcggggaccggcaggatgcctgcgagggcgacagtggggggcccatggtcgcctccttccacggcacctggttcctggtgggcctggtgagctggggtgagggctgtgggctccttcacaactacggcgtttacaccaaagtcagccgctacctcgactggatccatgggcacatcagagacaaggaagccccccagaagagctgggcaccttagcacccctccctgctcacctctggaccctagaagtcactcttggagtaaggctgggctagtgagtaccaagacagaggacattaaaggagcatgcaacaaacatacctccccgagtacctgtctgtcttttcatcctttttatgggctattctgggggaaagtaacattaattgagcatgcactacacaccaagtctatgaaaagaacctgcttaactcccaaagcagttgtgtagaagatctagtgggatctgagctgatatcacttctgggggtgagtggaggagattgatttagagaaaggaatttttttagaagttactgtaagagactaatagagcctttctcagggccttggaaagagcccgtgctagttacatcagaaaagcttgccagtgaccagtggccagtgagactcagaatggccatgtggtggagccaggattcaaaccaaggtcacactcccaaactcagctgcttctcttctttattatccctgggtgtgtgctggtgtgtgtgtgcgcgcgtgggtgtgtgggtggatacatgcatgtgtgtgtgtgtgtgtgtgtgtgtgtgtgtgtgtgtgtgtgttatatgtttggagaccagaggacaacttcgtttctcaacaccatccacttgttttgttttgtgttttgttttgtttgttgacacagggtctctcactgtcctgaaatctacccagtaggctaggctggctggctaccaaaccccaccccaccctggctttgacaagtggagacagaagaccagtagtccactggagatgtgaccagatgcccagaaggtgctcctcatggtgccctacagttttgttgaggagtctgtttaataatgcagctgggtgcagtggcagcacctgtagcccccaatactgaggcagcattgctgcagtctgagaggtggggctcgagggacctaataacttcgtatagcatacattatacgaagttatattaagggttccgcaagctctagtcgagccccagctggttctttccgcctcagaagccatagagcccaccgcatccccagcatgcctgctattgtcttcccaatcctcccccttgctgtcctgccccaccccaccccccagaatagaatgacacctactcagacaatgcgatgcaatttcctcattttattaggaaaggacagtgggagtggcaccttccagggtcaaggaaggcacgggggaggggcaaacaacagatggctggcaactagaaggcacagtcgaggctgatcagcgagctctagagaattgatcccctcagaagaactcgtcaagaaggcgatagaaggcgatgcgctgcgaatcgggagcggcgataccgtaaagcacgaggaagcggtcagcccattcgccgccaagctcttcagcaatatcacgggtagccaacgctatgtcctgatagcggtccgccacacccagccggccacagtcgatgaatccagaaaagcggccattttccaccatgatattcggcaagcaggcatcgccatgggtcacgacgagatcatcgccgtcgggcatgcgcgccttgagcctggcgaacagttcggctggcgcgagcccctgatgctcttcgtccagatcatcctgatcgacaagaccggcttccatccgagtacgtgctcgctcgatgcgatgtttcgcttggtggtcgaatgggcaggtagccggatcaagcgtatgcagccgccgcattgcatcagccatgatggatactttctcggcaggagcaaggtgagatgacaggagatcctgccccggcacttcgcccaatagcagccagtcccttcccgcttcagtgacaacgtcgagcacagctgcgcaaggaacgcccgtcgtggccagccacgatagccgcgctgcctcgtcctgcagttcattcagggcaccggacaggtcggtcttgacaaaaagaaccgggcgcccctgcgctgacagccggaacacggcggcatcagagcagccgattgtctgttgtgcccagtcatagccgaatagcctctccacccaagcggccggagaacctgcgtgcaatccatcttgttcaatggccgatcccatggtttagttcctcaccttgtcgtattatactatgccgatatactatgccgatgattaattgtcaacaggctgcaggtcgaaaggcccggagatgaggaagaggagaacagcgcggcagacgtgcgcttttgaagcgtgcagaatgccgggcctccggaggaccttcgggcgcccgccccgcccctgagcccgcccctgagcccgcccccggacccaccccttcccagcctctgagcccagaaagcgaaggagcaaagctgctattggccgctgccccaaaggcctacccgcttccattgctcagcggtgctgtccatctgcacgagactagtgagacgtgctacttccatttgtcacgtcctgcacgacgcgagctgcggggcgggggggaacttcctgactaggggaggagtagaaggtggcgcgaaggggccaccaaagaacggagccggttggcgcctaccggtggatgtggaatgtgtgcgaggccagaggccacttgtgtagcgccaagtgcccagcggggctgctaaagcgcatgctccagactgccttgggaaaagcgcctcccctacccggtagaatttcgacgacctgcagccaagctagcttcgcgagctcgaccgaacaaacgacccaacacccgtgcgttttattctgtctttttattgccgctcagctttacagtgacaatgacggctggcgactgaatattagtgcttacagacagcactacatattttccgtcgatgttgaaatcctttctcatatgtcaccataaatatcaaataattatagcaatcatttacgcgttaatggctaatcgccatcttccagcaggcgcaccattgcccctgtttcactatccaggttacggatatagttcatgacaatatttacattggtccagccaccagcttgcatgatctccggtattgaaactccagcgcgggccatatctcgcgcggctccgacacgggcactgtgtccagaccaggccaggtatctctgaccagagtcatccttagcgccgtaaatcaatcgatgagttgcttcaaaaatcccttccagggcgcgagttgatagctggctggtggcagatggcgcggcaacaccattttttctgacccggcaaaacaggtagttattcggatcatcagctacaccagagacggaaatccatcgctcgaccagtttagttacccccaggctaagtgccttctctacacctgcggtgctaaccagcgttttcgttctgccaatatggattaacattctcccaccgtcagtacgtgagatatctttaaccctgatcctggcaatttcggctatacgtaacagggtgttataagcaatccccagaaatgccagattacgtatatcctggcagcgatcgctattttccatgagtgaacgaacctggtcgaaatcagtgcgttcgaacgctagagcctgttttgcacgttcaccggcatcaacgttttcttttcggatccgccgcataaccagtgaaacagcattgctgtcacttggtcgtggcagcccggaccgacgatgaagcatgtttagctggcccaaatgttgctggatagtttttactgccagaccgcgcgcctgaagatatagaagataatcgcgaacatcttcaggttctgcgggaaaccatttccggttattcaacttgcaccatgccgcccacgaccggcaaacggacagaagcattttccaggtatgctcagaaaacgcctggcgatccctgaacatgtccatcaggttcttgcgaacctcatcactcgttgcatcgaccggtaatgcaggcaaattttggtgtacggtcagtaaattggacaccttcctcttcttcttgggcatggccgcaggaaagcagagccctgaagctcccatcaccggccaataagagccaagcctgcagtgtgacctcatagagcaatgtgccagccagcctgaccccaagggccctcaggcttgggcacactgtctctaggaccctgagagaaagacatacccatttctgcttagggccctgaggatgagcccaggggtggcttggcactgaagcaaaggacactggggctcagctggcagcaaagtgaccaggatgctgaggctttgacccagaagccagaggccagaggccaggacttctcttggtcccagtccaccctcactcagagctttaccaatgccctctggatagttgtcgggtaacggtggacgccactgattctctggccagcctaggacttcgccattccgctgattctgctcttccagccactggctgaccggttggaagtactccagcagtgccttggcatccagggcatctgagcctaccaggtccttcagtacctcctgccagggcctggagcagccagcctgcaacacctgcctgccaagcagagtgaccactgtgggcacaggggacacagggtggggcccacaacagcaccattgtccacttgtccctcactagtaaaagaactctagggttgcggggggtgggggaggtctctgtgaggctggtaagggatatttgcctggcccatggagctagcttggctggacgtaaactcctcttcagacctaataacttcgtatagcatacattatacgaagttatattaagggttattgaatatgatcggaattgggctgcaggaattcgatagcttggctgcaggtcgacgtacgtagcaagcttgatgggccctggtaccacagcctgggcaacacagcaaaaatcccttcccttaaaaaaaacaaaagagaaggaagaaggacgaagtagaatgtggaggacaaacaggggagagagggggaaagaaagggagggaattgtcttagagttttacggctgtgcacagacaccatgatcaaggtaactcttgtaaggataacatttagttggggctggcttacaggttcagaagttcagtccattatcatcaaggcaggaacatggcagcattcaaggcagacatggtgcaggaggagctgagagttctacatcttcatctgaagatttctagtagaatactggcttccaggcagctaggatgagggtcttaaagcccacacccagtgacacacctactccaacagggccacacctcctaatcatgccactccctgggctgagcatatagaaaccatcacagagtctaactagtgtggcccatcctgcacccatggaagaccatcactggggcatagacaacctccagagcccaccctgacagttcctgtctctgccttctccagcagtcaccagtttcaaatagctcctcaaggacagatggggccttgtgagcttcaccccgctgcaggctggaatgcgccacctttaatcccagcacttggaaggcagaggcaggcagatttctgagttcgaggccagcctagtctacagagtgagttccaggacagccagggcgatacagagaaaccctgtctcaaaaaacaaaacaaaacaaaacgatagaaaagagcaaagtgaccttgggctatggatgggatggaccatcgggcactgggttgggaagctgaactggtccagatgcccagagcccagagctctctcctcagcagttcataacctggggtgttgccacagcacacacagcaaggttagttctgctggttgtcgggacttagggtaggaggagtagaagcctgctactgattctgtctctctctgtttctctctcctccctccctccctccttccctccctccctccctcttcttcttcttctcatcctcctccctcttcctcttcttcctccacctccccaccccttattttgatacagggtttctctgtgtatccctggctgtcctggaactcactctgtagcccaggtgggcctcgaactctcagcctcagtccccagaatgctgagaacacaggtctgagtgatcactgatggctaaaagttgggattacattgttgttgcttgtttgtttattcttttgtacatgggacccaaatacaaatagtagcctcaacaataaacacgggataagttgctgctctgctttagggtctccctgacctctgtttttttgttttttgtttttggtatgttttgttttctgttgttgttgttatcatgtctataaatctatcttccttcctccctccttccttcccttcctacttccctctctttcttcatccctcccttccccctactctctttcacccccagataggaagcaagcatgataaaaacgtgtggtgttttcctttttatgtagagagtactgtgtagtgagtgttatcctatgggtgctgccattctgctgtatgttacctgctgtatgttataccaacctagatggtggtgaactcacatggttgcttccatcttggtgaggttaccagccaagatgtctgccctccacatgattgcctccatcttggtgaggtaaatgtttaataaagtaacaaaacaagacattaaaaacaaacattccagcacaaaatcttcttgagattagagacataataggaagtcaggtgaggtcatacaggccattaatcccatcacttggggaacagaggcaggtagaactttgaattgaaggcaggtatatttagtgatttccagggctatgtagagaggcccctgacccaactaataagtaaacaggaagataaataaatataatgaacttagaataaaacaaagaaaggaagaaacaagggaaggcagtgctgggggcctggcttatggtggatgggggaattctgtgctagggtgcctgaaactctgggctccatcctctgtagtgcataaactctttggtacgttagcccctgtctgtaacaaggagctgtccacggttgcagtactgcctttcccatctcagctgcccctcaggagctgtccacagtggcgacactttttcatcctcagcctacagctttagggaaacaccactgcaggggctgtcccaaaggtgctgtccacagaggcagcaccttctctgtggtctcacccctccagacaccccccagcagccccacagggatggcacctcagtaaaagccaactgtggccagagaagtcttcctaccctaactcatagactcgatgcagggaaaacagggtgaaaaaaagccaccaagccctgagctccccccagctcaggacttaaaatctcatcaatcctcactatggaaatctctgccttgagaagctctgccccctcataaatcctatataagaactgtccctttgtccagttccctgccatccgctcccaggagcagagggcagttatccctggattcatccctccacaccctggacctgccaataaacctttcttgagatttcatgcttcctgtgattctcagtggaagaagccaagaagaaaagaaccaaagagagggagccaggctgaggctcctgagttcttcagctcagctgtggatacctgtgatggtttgtatatgctctgtccagggaatggcatgattagaaggtgtggccctgttgaagtaggtgtgtcactgtgggtgtgggctataagaccctcatcttaactgcatggaagtcattcttccactggcagccttcagatgaaaatgtagaactctcagctcctcctgcaccatgcctgcctagatgctgccctgctcccaccttgatgataatggactgaacctctgaacctgtaagccagccccaattaaatgttgttctttataagtcttgccttggttgtggtgtctgttcacagcagtaaaaccatgactaagacaatatcttctacttggagctgcaacaactctgctgaggaggcttcctctcagagctatatggttcctggtatctgtaaaattcccttctattgggacactttccaacctcagatctgtgtggttcctggcccctgtgtctcgggatgcccttccattagaacagcttctcccctcagagctgcatggttcctggacttctgagtcccaggagacccttccatctgagcagaaacacttacaggagcagagtcctccaacaccacggttttgttttgaaagaccaagaccaaccctcaggaggtttctggcaaaggcagattctaggtgcacctggaggagacctatagtgcaggaccatccgtcgtaggttgctaggcaccaatgggcaaaggtagggaagaaatcttaccagaagattctattccattccattctcctcacaatgtaagagccaaagttaacctctaaggcccaagaacaaggtaactctccagaatgctgggagatgtagttcttgggtaacaacaagccatgttctcgccctaaacaagtttgtttgaatcaactacactgaatgtacttgatcatatgtaggagagagaagattgattctagttcagggtttcaggctatttcagtccaccatgatgggaaaggcatgacattgtttatgacagtaagagcatgtagcagaggatcctcacatcacaacaggccgaaatgcagaggacagtgcaaccagaggacagtctgtaactttccaagtccctcttctagtgggttgcttccaccacctctcaggtggtgctacagctcaggaacaattgagatgtgtgatgaagggcaggtactcaactgtggctgtattgtatccttttatagttgtcctctgtgtgttgagctatgtgcgagattctcaggtcatcggagtacctgttttactttggcaggcataggagactcctgagaactctgcctgacatccttgccagcccaagctttggtttagtgtgtgcagtatcactcttgggtcttatctgcatatccctgatggcccatcaagatgtgt

SEQ ID NO: 10 - DNA, 1386 bp, Mouse
atgtggcaattcagagtcttcctgctgctcatgtccacctggggaatatctagcataccggcccatcctgacccagtgttctccagcagcgagcatgcccaccaggtgcttcgggtcagacgtgccaacagcttcctggaagagatgcggccaggcagcctggaacgggagtgtatggaggagatctgtgacttcgaggaggcccaggagattttccaaaatgtggaagacacactggccttctggatcaagtactttgacggtgaccagtgctcggctccacccttggaccaccagtgcgacagcccatgctgcgggcatggcacttgcatcgacggcataggcagcttcagctgcagctgcgataagggctgggagggcaagttctgtcagcaggagttgcgcttccaggactgtcgggtgaacaatggcggctgcttgcactactgcctggaggagagcaatgggcggcgctgcgcttgtgccccgggctatgagctggcagacgaccacatgcgctgcaagtccactgtgaattttccatgtgggaaactggggaggtggatagagaagaaacgcaagatcctcaaacgagacacagacttagaagatgaactggaaccagatccaaggatagtcaacggaacgctgacgaagcagggtgacagtccttggcaggcaatccttctggactccaagaagaagctggcctgcggaggggtgctcatccacacttcctgggtgctgacggcagcccactgcgtggagggcaccaagaagcttaccgtgaggcttggtgagtatgatctgcgacgcagggaccactgggagctggacctggacatcaaggagatcctcgtccaccctaactacacccggagcagcagtgacaacgacattgctctgctccgcctagcccagccagccactctctccaaaaccatagtgcccatctgcctgccgaacaatgggctcgctcagcaggagctcactcaggctggccaggagacagtggtgacaggctggggctatcaaagcgacagaatcaaggatggcagaaggaaccgcaccttcatcctcaccttcatccgcatccctttggttgctcgaaatgagtgcgtggaggtcatgaagaatgtggtctcggagaacatgctgtgtgcaggcatcattgggaacacgagagacgcctgtgatggtgacagtggggggcccatggtggtcttctttcggggtacctggttcctggtgggcctggtgagctggggtgagggctgtgggcacaccaacaactatggcatctacaccaaagtgggaagctacctcaaatggattcacagttacattggggaaaagggtgtctcccttaagagccagaagctatag

SEQ ID NO: 11 - protein, 461 aa, Human
MWQLTSLLLFVATWGISGTPAPLDSVFSSSERAHQVLRIRKRANSFLEELRHSSLERECIEEICDFEEAKEIFQNVDDTLAFWSKHVDGDQCLVLPLEHPCASLCCGHGTCIDGIGSFSCDCRSGWEGRFCQREVSFLNCSLDNGGCTHYCLEEVGWRRCSCAPGYKLGDDLLQCHPAVKFPCGRPWKRMEKKRSHLKRDTEDQEDQVDPRLIDGKMTRRGDSPWQVVLLDSKKKLACGAVLIHPSWVLTAAHCMDESKKLLVRLGEYDLRRWEKWELDLDIKEVFVHPNYSKSTTDNDIALLHLAQPATLSQTIVPICLPDSGLAERELNQAGQETLVTGWGYHSSREKEAKRNRTFVLNFIKIPVVPHNECSEVMSNMVSENMLCAGILGDRQDACEGDSGGPMVASFHGTWFLVGLVSWGEGCGLLHNYGVYTKVSRYLDWIHGHIRDKEAPQKSWAP

SEQ ID NO: 12 - protein, 461 aa, Mouse
MWQFRVFLLLMSTWGISSIPAHPDPVFSSSEHAHQVLRVRRANSFLEEMRPGSLERECMEEICDFEEAQEIFQNVEDTLAFWIKYFDGDQCSAPPLDHQCDSPCCGHGTCIDGIGSFSCSCDKGWEGKFCQQELRFQDCRVNNGGCLHYCLEESNGRRCACAPGYELADDHMRCKSTVNFPCGKLGRWIEKKRKILKRDTDLEDELEPDPRIVNGTLTKQGDSPWQAILLDSKKKLACGGVLIHTSWVLTAAHCVEGTKKLTVRLGEYDLRRRDHWELDLDIKEILVHPNYTRSSSDNDIALLRLAQPATLSKTIVPICLPNNGLAQQELTQAGQETVVTGWGYQSDRIKDGRRNRTFILTFIRIPLVARNECVEVMKNVVSENMLCAGIIGNTRDACDGDSGGPMVVFFRGTWFLVGLVSWGEGCGHTNNYGIYTKVGSYLKWIHSYIGEKGVSLKSQKL

SEQ ID NO: 13 - DNA, 24 bp, Artificial Sequence
  Neo-F (P1) primer
aggctggtaagggatatttgcctg

SEQ ID NO: 14 - DNA, 24 bp, Artificial Sequence
  3'arm-R (P2) primer
gagtgagcccagacccataacaat

SEQ ID NO: 15 - DNA, 25 bp, Artificial Sequence
  5'arm-F (P3) primer
tgggattacaagaaacgcctcagac

SEQ ID NO: 16 - DNA, 22 bp, Artificial Sequence
  KI-R (P4) primer
aggagttggcacgtttgcggat

SEQ ID NO: 17 - DNA, 25 bp, Artificial Sequence
  KI-F (F1) primer
tgggattacaagaaacgcctcagac

SEQ ID NO: 18 - DNA, 22 bp, Artificial Sequence
  KI-R (R1) primer
aggagttggcacgtttgcggat

SEQ ID NO: 19 - DNA, 24 bp, Artificial Sequence
  KI2-F (F2) primer
ggctgtgggctccttcacaactac

SEQ ID NO: 20 - DNA, 27 bp, Artificial Sequence
  KI2-R (R2) primer
caggttcttttcatagacttggtgtgt

SEQ ID NO: 21 - DNA, 24 bp, Artificial Sequence
  Neo-del-F (F3) primer
agggacctaataacttcgtatagc

SEQ ID NO: 22 - DNA, 24 bp, Artificial Sequence
  Neo-del-R (R3) primer
cctgtttgtcctccacattctact

SEQ ID NO: 23 - DNA, 22 bp, Artificial Sequence
  WT-F (F4) primer
catctacaccaaagtgggaagc

SEQ ID NO: 24 - DNA, 27 bp, Artificial Sequence
  KI2-R (R2) primer
caggttcttttcatagacttggtgtgt

SEQ ID NO: 25 - DNA, 25 bp, Artificial Sequence
  Seq-F (F1) primer
tgggattacaagaaacgcctcagac

SEQ ID NO: 26 - DNA, 24 bp, Artificial Sequence
  Seq-R (R3) primer
cctgtttgtcctccacattctact

SEQ ID NO: 27 - DNA, 25 bp, Artificial Sequence
  hproC 1-F primer
tgggattacaagaaacgcctcagac

SEQ ID NO: 28 - DNA, 22 bp, Artificial Sequence
  hproC 1-R primer
aggagttggcacgtttgcggat

SEQ ID NO: 29 - DNA, 22 bp, Artificial Sequence
  mproC -F primer
catctacaccaaagtgggaagc

SEQ ID NO: 30 - DNA, 27 bp, Artificial Sequence
  mproC -R primer
caggttcttttcatagacttggtgtgt

SEQ ID NO: 31 - DNA, 20 bp, Artificial Sequence
  F8-Common primer
gagcaaattcctgtactgac

SEQ ID NO: 32 - DNA, 20 bp, Artificial Sequence
  F8-WT-Forward primer
tgcaaggcctgggcttattt

SEQ ID NO: 33 - DNA, 20 bp, Artificial Sequence
  F8-Mut-Forward primer
tgtgtcccgccccttccttt

SEQ ID NO: 34 - DNA, 23 bp, Artificial Sequence
  F9-Common primer
aacagggatagtaagattgttcc

SEQ ID NO: 35 - DNA, 22 bp, Artificial Sequence
  F9-WT primer
tggaagcagtatgttggtaagc

SEQ ID NO: 36 - DNA, 21 bp, Artificial Sequence
  F9-Mut primer
tcctgtcatctcaccttgctc